European Patent Specification EP 3 777 877 B1, published August 7, 2024. Title: ADMINISTRATION OF AN ANTAGONIST OF ALPHA5BETA1 FOR ANTI-ANGIOGENESIS AND CANCER TREATMENT. Applicant: FENG, XIAODONG. Application 13/374,369. The sequence listing filed with the application follows.

SEQUENCE LISTING (6 sequences)

SEQ ID NO: 1 - protein, 65 aa, Vipera lebetina
MNSGNPCCDPVTCKPRRGEHCVSGPCCRNCKFLNAGTICKRARGDDMNDYCTGISPDCPRNPWKG

SEQ ID NO: 2 - protein, 137 aa, Vipera palestinae
  MOD_RES (99)..(124): Any amino acid
  MOD_RES (134)..(137): Any amino acid
DQDCLPGWSFYEGNCYKAFDEPKSWVDAEKFCQKQSNGKHLASIEGLGKANFVAKLVSEDQSETLREPQIHVWIGLRDQSERQQCSSHWTDGSAVSYEXXXXXXXXXXXXXXXXXXXXXXXXXXCGLAYPFICXXXX

SEQ ID NO: 3 - protein, 125 aa, Vipera palestinae
DQDCLPGWSYFEKYCYKVFQVKKNWEDAEKFCTEEVKDGHLISLHSNEEVEFMTSLAFPILKYDIVWMGLRNFWRDCPWKWSDDAKLDYKAWSDEPNCYGAMTTDYQWLRWNCNDPRYFVCKSPA

SEQ ID NO: 4 - protein, 49 aa, Echis carinatus
QCESGPCCRNCKFLKEGTICKRARGDDMDDYCNGKTCDCPRNPHKGPAT

SEQ ID NO: 5 - protein, 10 aa, Artificial Sequence
  Description of Artificial Sequence: Synthetic peptide
  MOD_RES (2)..(2): Pen
GXGRGDSPCA

SEQ ID NO: 6 - protein, 6 aa, Artificial Sequence
  Description of Artificial Sequence: Synthetic peptide
GRGESP